European Patent Specification EP 4 041 748 B1, published May 1, 2024. Title: Peptide compounds for reducing side effects of CB1 receptor agonists. Applicant: UNIVERSITAT DE BARCELONA UNIVERSITAT POMPEU FABRA UNIVERISTAT AUTÒNOMA DE BARCELONA INSTITUTO DE MEDICINA MOLECULAR JOÃO LOBO ANTU. The sequence listing filed with the application follows.

SEQUENCE LISTING (2 sequences)

SEQ ID NO: 1 - protein, 37 aa, Artificial Sequence
  Transmembrane region 5 of cannabinoid receptor 1 (TM5)
ETYLMFWIGVTSVLLLFIVYAYMYILWGRKKRRQRRR

SEQ ID NO: 2 - protein, 10 aa, Artificial Sequence
  Cell penetrating peptidic sequence Tat
GRKKRRQRRR